European Patent Specification EP 3 158 077 B1, published April 5, 2023. Title: CELL CULTURE METHODS AND MEDIA COMPRISING N-ACETYLCYSTEINE. Applicant: HOLMAN, BRENA LEE, JEONG. The sequence listing filed with the application follows.

SEQUENCE LISTING (32 sequences)

SEQ ID NO: 1 - protein, 122 aa, Artificial Sequence
  Description of Artificial Sequence: Synthetic polypeptide
QVQLVQSGAEVKKPGASVKVSCKASGYTFTNYGLSWVRQAPGQGLEWMGWISANNGDTNYGQEFQGRVTMTTDTSTSTAYMELRSLRSDDTAVYYCARDSSSSWARWFFDLWGRGTLVTVSS

SEQ ID NO: 2 - protein, 108 aa, Artificial Sequence
  Description of Artificial Sequence: Synthetic polypeptide
SYVLTQPPSVSVAPGKTARITCGGNIIGSKLVHWYQQKPGQAPVLVIYDDGDRPSGIPERFSGSNSGNTATLTISRVEAGDEADYYCQVWDTGSDPVVFGGGTKLTVL

SEQ ID NO: 3 - protein, 5 aa, Artificial Sequence
  Description of Artificial Sequence: Synthetic peptide
NYGLS

SEQ ID NO: 4 - protein, 17 aa, Artificial Sequence
  Description of Artificial Sequence: Synthetic peptide
WISANNGDTNYGQEFQG

SEQ ID NO: 5 - protein, 13 aa, Artificial Sequence
  Description of Artificial Sequence: Synthetic peptide
DSSSSWARWFFDL

SEQ ID NO: 6 - protein, 11 aa, Artificial Sequence
  Description of Artificial Sequence: Synthetic peptide
GGNIIGSKLVH

SEQ ID NO: 7 - protein, 7 aa, Artificial Sequence
  Description of Artificial Sequence: Synthetic peptide
DDGDRPS

SEQ ID NO: 8 - protein, 11 aa, Artificial Sequence
  Description of Artificial Sequence: Synthetic peptide
QVWDTGSDPVV

SEQ ID NO: 9 - protein, 122 aa, Artificial Sequence
  Description of Artificial Sequence: Synthetic polypeptide
EVQLVQSGAEVKKPGASVKVSCKASGYTFRNYGLSWVRQAPGQGLEWMGWISANNGDTNYGQEFQGRITMTTETSTNTAHMELRSLRSDDTAVYYCVRDSSSNWARWFFDLWGKGTMVTVSS

SEQ ID NO: 10 - protein, 108 aa, Artificial Sequence
  Description of Artificial Sequence: Synthetic polypeptide
SYVLTQPPSVSVAPGQTARIPCGGNNIGSKLVHWYQQKPGQAPVLVVYDDGDRPSGIPERFSGSNSGNTATLTISRIDAGDEADYYCQVWDTGSDPVVFGGGTKLTVL

SEQ ID NO: 11 - protein, 5 aa, Artificial Sequence
  Description of Artificial Sequence: Synthetic peptide
NYGLS

SEQ ID NO: 12 - protein, 17 aa, Artificial Sequence
  Description of Artificial Sequence: Synthetic peptide
WISANNGDTNYGQEFQG

SEQ ID NO: 13 - protein, 13 aa, Artificial Sequence
  Description of Artificial Sequence: Synthetic peptide
DSSSNWARWFFDL

SEQ ID NO: 14 - protein, 11 aa, Artificial Sequence
  Description of Artificial Sequence: Synthetic peptide
GGNNIGSKLVH

SEQ ID NO: 15 - protein, 7 aa, Artificial Sequence
  Description of Artificial Sequence: Synthetic peptide
DDGDRPS

SEQ ID NO: 16 - protein, 11 aa, Artificial Sequence
  Description of Artificial Sequence: Synthetic peptide
QVWDTGSDPVV

SEQ ID NO: 17 - protein, 122 aa, Artificial Sequence
  Description of Artificial Sequence: Synthetic polypeptide
QVQLVQSGAEVKKPGASVKVSCKASGYTFTNYGLSWVRQAPGQGLEWMGWINYDGGNTQYGQEFQGRVTMTTDTSTSTAYMELRSLRSDDTAVYYCARDSSSSWARWFFDLWGRGTLVTVSS

SEQ ID NO: 18 - protein, 108 aa, Artificial Sequence; identical to SEQ ID NO: 2
  Description of Artificial Sequence: Synthetic polypeptide

SEQ ID NO: 19 - protein, 5 aa, Artificial Sequence
  Description of Artificial Sequence: Synthetic peptide
NYGLS

SEQ ID NO: 20 - protein, 17 aa, Artificial Sequence
  Description of Artificial Sequence: Synthetic peptide
WINYDGGNTQYGQEFQG

SEQ ID NO: 21 - protein, 13 aa, Artificial Sequence
  Description of Artificial Sequence: Synthetic peptide
DSSSSWARWFFDL

SEQ ID NO: 22 - protein, 11 aa, Artificial Sequence
  Description of Artificial Sequence: Synthetic peptide
GGNIIGSKLVH

SEQ ID NO: 23 - protein, 7 aa, Artificial Sequence
  Description of Artificial Sequence: Synthetic peptide
DDGDRPS

SEQ ID NO: 24 - protein, 11 aa, Artificial Sequence
  Description of Artificial Sequence: Synthetic peptide
QVWDTGSDPVV

SEQ ID NO: 25 - protein, 122 aa, Artificial Sequence
  Description of Artificial Sequence: Synthetic polypeptide
QVQLVQSGAEVKKPGASVKVSCKASGYTFEQTGVSWVRQAPGQGLEWMGWISANNGDTNYGQEFQGRVTMTTDTSTSTAYMELRSLRSDDTAVYYCARDSSSSWARWFFDLWGRGTLVTVSS

SEQ ID NO: 26 - protein, 108 aa, Artificial Sequence; identical to SEQ ID NO: 2
  Description of Artificial Sequence: Synthetic polypeptide

SEQ ID NO: 27 - protein, 5 aa, Artificial Sequence
  Description of Artificial Sequence: Synthetic peptide
QTGVS

SEQ ID NO: 28 - protein, 17 aa, Artificial Sequence
  Description of Artificial Sequence: Synthetic peptide
WISANNGDTNYGQEFQG

SEQ ID NO: 29 - protein, 13 aa, Artificial Sequence
  Description of Artificial Sequence: Synthetic peptide
DSSSSWARWFFDL

SEQ ID NO: 30 - protein, 11 aa, Artificial Sequence
  Description of Artificial Sequence: Synthetic peptide
GGNIIGSKLVH

SEQ ID NO: 31 - protein, 7 aa, Artificial Sequence
  Description of Artificial Sequence: Synthetic peptide
DDGDRPS

SEQ ID NO: 32 - protein, 11 aa, Artificial Sequence
  Description of Artificial Sequence: Synthetic peptide
QVWDTGSDPVV